European Patent Application EP 4 112 072 A1, published January 4, 2023. Title: RECOMBINANT HVT VECTORS EXPRESSING MULTIPLE ANTIGENS OF AVIAN PATHOGENS, AND VACCINES COMPRISING THEM. Applicant: Boehringer Ingelheim Animal Health USA Inc. Application EP 17823319.3. The sequence listing filed with the application follows.

SEQUENCE LISTING (27 sequences)

SEQ ID NO: 1 - DNA, 1359 bp, artificial sequence
  DNA encoding IBDV VP2
atgacaaacctgcaagatcaaacccaacagattgttccgttcatacggagccttctgatgccaacaaccggaccggcgtccattccggacgacaccctggagaagcacactctcaggtcagagacctcgacctacaatttgactgtgggggacacagggtcagggctaattgtctttttccctggattccctggctcaattgtgggtgctcactacacactgcagagcaatgggaactacaagttcgatcagatgctcctgactgcccagaacctaccggccagctacaactactgcagactagtgagtcggagtctcacagtgaggtcaagcacactccctggtggcgtttatgcactaaacggcaccataaacgccgtgaccttccaaggaagcctgagtgaactgacagatgttagctacaatgggttgatgtctgcaacagccaacatcaacgacaaaattgggaatgtcctggtaggggaaggggtcactgtcctcagcctacccacatcatatgatcttgggtatgtgaggcttggtgaccccattcccgctatagggcttgacccaaaaatggtagctacatgcgacagcagtgacaggcccagagtctacaccataactgcagccgatgattaccaattctcatcacagtaccaaccaggtggggtaacaatcacactgttctcagccaacattgatgctatcacaagcctcagcattgggggagagctcgtgtttcaaacaagcgtccaaggccttgtactgggcgccaccatctaccttataggctttgatgggactgcggtaatcaccagagctgtagccgcagataatgggctgacggccggcaccgacaatcttatgccattcaatcttgtcattccaaccaatgagataacccagccaatcacatccatcaaactggagatagtgacctccaaaagtggtggtcaggcaggggatcagatgtcatggtcggcaagtgggagcctagcagtgacgatccatggtggcaactatccaggggccctccgtcccgtcacactagtagcctacgaaagagtggcaacaggatccgtcgttacggtcgctggggtgagtaacttcgagctgattccaaatcctgaactagcaaagaacctggttacagaatacggccgatttgacccaggagccatgaactacacaaaattgatactgagtgagagggaccgtcttggcatcaagaccgtctggccaacaagggagtacactgattttcgtgagtacttcatggaggtggccgacctcaactctcccctgaagattgcaggagcatttggcttcaaagacataatccgggctataaggagg

SEQ ID NO: 2 - protein, 453 aa, artificial sequence
  IBDV VP2 protein
MTNLQDQTQQIVPFIRSLLMPTTGPASIPDDTLEKHTLRSETSTYNLTVGDTGSGLIVFFPGFPGSIVGAHYTLQSNGNYKFDQMLLTAQNLPASYNYCRLVSRSLTVRSSTLPGGVYALNGTINAVTFQGSLSELTDVSYNGLMSATANINDKIGNVLVGEGVTVLSLPTSYDLGYVRLGDPIPAIGLDPKMVATCDSSDRPRVYTITAADDYQFSSQYQPGGVTITLFSANIDAITSLSIGGELVFQTSVQGLVLGATIYLIGFDGTAVITRAVAADNGLTAGTDNLMPFNLVIPTNEITQPITSIKLEIVTSKSGGQAGDQMSWSASGSLAVTIHGGNYPGALRPVTLVAYERVATGSVVTVAGVSNFELIPNPELAKNLVTEYGRFDPGAMNYTKLILSERDRLGIKTVWPTREYTDFREYFMEVADLNSPLKIAGAFGFKDIIRAIRR

SEQ ID NO: 3 - DNA, 1659 bp, artificial sequence
  NDV-Fopt VIId of pFSV40VP2 and pFIRESVP2
atgggcagcaagcccagcacaagaatcccagcccccctgatgctgatcacccgcatcatgctgatcctgggctgcatcagacccacaagctccctggatggacgccccctggccgctgccggcatcgtggtgaccggcgacaaggccgtgaacgtgtacaccagcagccagaccggcagcatcatcgtgaagctgctgcccaacatgcccagagacaaagaggcctgcgccaaggcccccctggaagcctacaacagaaccctgaccaccctgctgacccccctgggcgacagcatcagaaagatccagggctccgtgagcacaagcggcggaggaaagcagggcagactgatcggcgccgtgatcggcagcgtggccctgggagtggctacagctgcccagattaccgctgcagccgccctgatccaggccaaccagaacgccgccaacatcctgagactgaaagagagcattgccgccaccaacgaggccgtgcacgaagtgaccgacggcctgagccagctgtccgtggccgtgggcaagatgcagcagttcgtgaacgaccagttcaacaacaccgccagagagctggactgcatcaagatcacccagcaggtgggcgtggagctgaacctgtacctgaccgagctgaccacagtgttcggcccccagatcacaagcccagccctgacacagctgaccatccaggccctgtacaacctggctggcggcaacatggactatctgctgacaaagctgggaatcggcaacaaccagctgtccagcctgatcggaagcggcctgatcaccggctaccccatcctgtacgacagccagacacagctgctgggcatccaggtgaacctgcccagcgtgggcaacctgaacaacatgcgcgccacctacctggaaaccctgagcgtgtccaccaccaagggctacgccagcgccctggtgcccaaggtggtgacacaggtgggcagcgtgatcgaggaactggacaccagctactgcatcgagagcgacctggacctgtactgcaccagaatcgtgaccttcccaatgagccccggcatctacagctgcctgagcggcaacaccagcgcctgcatgtacagcaagaccgaaggcgcactgacaacaccctacatggccctgaagggaagcgtgatcgccaactgcaagatcaccacctgcagatgcaccgaccccccaggcatcatcagccagaactacggcgaggccgtgagcctgatcgatcgccattcctgtaacgtgctgtccctggacggcatcacactgagactgagcggcgagttcgatgccacctaccagaagaacatcagcatcctggacagccaggtgatcgtgaccggcaacctggacatcagcaccgagctgggcaacgtgaataacagcatcagcaacgccctggacagactggccgagagcaacagcaagctggaaaaagtgaacgtgcgcctgacatccacttccgctctgatcacctacatcgtgctgaccgtgatcagcctggtgttcggcgccctgagcctggtgctggcctgctacctgatgtacaagcagaaggcccagcagaaaaccctgctgtggctgggcaacaacaccctggaccagatgagagccaccaccagagcc

SEQ ID NO: 4 - DNA, 1659 bp, artificial sequence
  NDV-F wildtype VIId of pFP2AVP2
atgggctccaaaccttctaccaggatcccagcacctctgatgctgatcacccggattatgctgatattgggctgtatccgtccgacaagctctcttgacggcaggcctcttgcagctgcaggaattgtagtaacaggagataaggcagtcaatgtatacacttcgtctcagacagggtcaatcatagtcaagttgctcccgaatatgcccagggataaggaggcgtgtgcaaaagccccattagaggcatataacagaacactgactactttgctcactcctcttggcgactccatccgcaagatccaagggtctgtgtccacatctggaggaggcaagcaaggccgcctgataggtgctgttattggcagtgtagctcttggggttgcaacagcggcacagataacagcagctgcggccctaatacaagccaaccagaatgccgccaacatcctccggcttaaggagagcattgctgcaaccaatgaagctgtgcatgaagtcaccgacggattatcacaactatcagtggcagttgggaagatgcagcagtttgtcaatgaccagtttaataatacggcgcgagaattggactgtataaaaatcacacaacaggttggtgtagaactcaacctatacctaactgaattgactacagtattcgggccacagatcacctcccctgcattaactcagctgaccatccaggcactttataatttagctggtggcaatatggattacttattaactaagttaggtatagggaacaatcaactcagctcgttaattggtagcggcctgatcactggttaccctatactgtatgactcacagactcaactcttgggcatacaagtgaatttaccctcagtcgggaacttaaataatatgcgtgccacctatttggagaccttatctgtaagtacaaccaaaggatatgcctcagcacttgtcccgaaagtagtgacacaagtcggttccgtgatagaagagcttgacacctcatactgtatagagtccgatctggatttatattgtactagaatagtgacattccccatgtccccaggtatttattcctgtttgagcggcaacacatcagcttgcatgtattcaaagactgaaggcgcactcactacgccgtatatggcccttaaaggctcagttattgccaattgtaaaataacaacatgtagatgtacagaccctcctggtatcatatcgcaaaattatggagaagctgtatccctgatagatagacattcgtgcaatgtcttatcattagacgggataactctaaggctcagtggggaatttgatgcaacttatcaaaagaacatctcaatactagattctcaagtcatcgtgacaggcaatcttgatatatcaactgaacttggaaacgtcaacaattcaatcagcaatgccttggataggttggcagaaagcaacagcaagctagaaaaagtcaatgtcagactaaccagcacatctgctctcattacctatattgttctaactgtcatttctctagttttcggtgcacttagtctggtgttagcgtgttacctgatgtacaaacagaaggcacaacaaaagaccttgctatggcttgggaataataccctcgatcagatgagagccactacaagagca

SEQ ID NO: 5 - protein, 553 aa, artificial sequence
  NDV-F VIId
MGSKPSTRIPAPLMLITRIMLILGCIRPTSSLDGRPLAAAGIVVTGDKAVNVYTSSQTGSIIVKLLPNMPRDKEACAKAPLEAYNRTLTTLLTPLGDSIRKIQGSVSTSGGGKQGRLIGAVIGSVALGVATAAQITAAAALIQANQNAANILRLKESIAATNEAVHEVTDGLSQLSVAVGKMQQFVNDQFNNTARELDCIKITQQVGVELNLYLTELTTVFGPQITSPALTQLTIQALYNLAGGNMDYLLTKLGIGNNQLSSLIGSGLITGYPILYDSQTQLLGIQVNLPSVGNLNNMRATYLETLSVSTTKGYASALVPKVVTQVGSVIEELDTSYCIESDLDLYCTRIVTFPMSPGIYSCLSGNTSACMYSKTEGALTTPYMALKGSVIANCKITTCRCTDPPGIISQNYGEAVSLIDRHSCNVLSLDGITLRLSGEFDATYQKNISILDSQVIVTGNLDISTELGNVNNSISNALDRLAESNSKLEKVNVRLTSTSALITYIVLTVISLVFGALSLVLACYLMYKQKAQQKTLLWLGNNTLDQMRATTRA

SEQ ID NO: 6 - DNA, 1391 bp, artificial sequence
  mCMV IE promoter
aactccgcccgttttatgactagaaccaatagtttttaatgccaaatgcactgaaatcccctaatttgcaaagccaaacgccccctatgtgagtaatacggggactttttacccaatttcccaagcggaaagccccctaatacactcatatggcatatgaatcagcacggtcatgcactctaatggcggcccatagggactttccacatagggggcgttcaccatttcccagcataggggtggtgactcaatggcctttacccaagtacattgggtcaatgggaggtaagccaatgggtttttcccattactggcaagcacactgagtcaaatgggactttccactgggttttgcccaagtacattgggtcaatgggaggtgagccaatgggaaaaacccattgctgccaagtacactgactcaatagggactttccaatgggtttttccattgttggcaagcatataaggtcaatgtgggtgagtcaatagggactttccattgtattctgcccagtacataaggtcaatagggggtgaatcaacaggaaagtcccattggagccaagtacactgcgtcaatagggactttccattgggttttgcccagtacataaggtcaataggggatgagtcaatgggaaaaacccattggagccaagtacactgactcaatagggactttccattgggttttgcccagtacataaggtcaatagggggtgagtcaacaggaaagtcccattggagccaagtacattgagtcaatagggactttccaatgggttttgcccagtacataaggtcaatgggaggtaagccaatgggtttttcccattactggcacgtatactgagtcattagggactttccaatgggttttgcccagtacataaggtcaataggggtgaatcaacaggaaagtcccattggagccaagtacactgagtcaatagggactttccattgggttttgcccagtacaaaaggtcaatagggggtgagtcaatgggtttttcccattattggcacgtacataaggtcaataggggtgagtcattgggtttttccagccaatttaattaaaacgccatgtactttcccaccattgacgtcaatgggctattgaaactaatgcaacgtgacctttaaacggtactttcccatagctgattaatgggaaagtaccgttctcgagccaatacacgtcaatgggaagtgaaagggcagccaaaacgtaacaccgccccggttttcccctggaaattccatattggcacgcattctattggctgagctgcgttctacgtgggtataagaggcgcgaccagcgtcggtaccgtcgcagtcttcggtctgaccaccgtagaacgcagagctcctcgctgcag

SEQ ID NO: 7 - DNA, 345 bp, artificial sequence
  SV40 Promoter for NDV F
gctgtggaatgtgtgtcagttagggtgtggaaagtccccaggctccccagcaggcagaagtatgcaaagcatgcatctcaattagtcagcaaccaggtgtggaaagtccccaggctccccagcaggcagaagtatgcaaagcatgcatctcaattagtcagcaaccatagtcccgcccctaactccgcccatcccgcccctaactccgcccagttccgcccattctccgccccatggctgactaattttttttatttatgcagaggccgaggccgcctcggcctctgagctattccagaagtagtgaggaggcttttttggaggcctaggcttttgcaaaaagct

SEQ ID NO: 8 - DNA, 199 bp, artificial sequence
  SV40 Poly A
ggggatccagacatgataagatacattgatgagtttggacaaaccacaactagaatgcagtgaaaaaaatgctttatttgtgaaatttgtgatgctattgctttatttgtaaccattataagctgcaataaacaagttaacaacaacaattgcattcattttatgtttcaggttcagggggaggtgtgggaggtttttt

SEQ ID NO: 9 - DNA, 154 bp, artificial sequence
  Synthetic Poly A
aataaaatatctttattttcattacatctgtgtgttggttttttgtgtgaatcgatagtactaacatacgctctccatcaaaacaaaacgaaacaaaacaaactagcaaaataggctgtccccagtgcaagtgcaggtgccagaacatttctct

SEQ ID NO: 10 - DNA, 563 bp, artificial sequence
  IRES of pFIRESVP2
cccccccccctaacgttactggccgaagccgcttggaataaggccggtgtgcgtttgtctatatgttattttccaccatattgccgtcttttggcaatgtgagggcccggaaacctggccctgtcttcttgacgagcattcctaggggtctttcccctctcgccaaaggaatgcaaggtctgttgaatgtcgtgaaggaagcagttcctctggaagcttcttgaagacaaacaacgtctgtagcgaccctttgcaggcagcggaaccccccacctggcgacaggtgcctctgcggccaaaagccacgtgtataagatacacctgcaaaggcggcacaaccccagtgccacgttgtgagttggatagttgtggaaagagtcaaatggctctcctcaagcgtattcaacaaggggctgaaggatgcccagaaggtaccccattgtatgggatctgatctggggcctcggtgcacatgctttacatgtgtttagtcgaggttaaaaaacgtctaggccccccgaaccacggggacgtggttttcctttgaaaaacacgatgataat

SEQ ID NO: 11 - DNA, 66 bp, artificial sequence
  P2A of pFP2AVP2
ggctccggcgccaccaacttctccctgctcaagcaggccggcgacgtggaggagaaccctggacct

SEQ ID NO: 12 - DNA, 3807 bp, artificial sequence
  pFSV40VP2 for vHVT309
  IBDV VP2 (1)..(1362)
  SV40 Poly A (1383)..(1594)
  SV40 Promoter (1624)..(1968)
  NDV-Fopt VIId (1981)..(3645)
  Synthetic Poly A (3654)..(3807)
atgacaaacctgcaagatcaaacccaacagattgttccgttcatacggagccttctgatgccaacaaccggaccggcgtccattccggacgacaccctggagaagcacactctcaggtcagagacctcgacctacaatttgactgtgggggacacagggtcagggctaattgtctttttccctggattccctggctcaattgtgggtgctcactacacactgcagagcaatgggaactacaagttcgatcagatgctcctgactgcccagaacctaccggccagctacaactactgcagactagtgagtcggagtctcacagtgaggtcaagcacactccctggtggcgtttatgcactaaacggcaccataaacgccgtgaccttccaaggaagcctgagtgaactgacagatgttagctacaatgggttgatgtctgcaacagccaacatcaacgacaaaattgggaatgtcctggtaggggaaggggtcactgtcctcagcctacccacatcatatgatcttgggtatgtgaggcttggtgaccccattcccgctatagggcttgacccaaaaatggtagctacatgcgacagcagtgacaggcccagagtctacaccataactgcagccgatgattaccaattctcatcacagtaccaaccaggtggggtaacaatcacactgttctcagccaacattgatgctatcacaagcctcagcattgggggagagctcgtgtttcaaacaagcgtccaaggccttgtactgggcgccaccatctaccttataggctttgatgggactgcggtaatcaccagagctgtagccgcagataatgggctgacggccggcaccgacaatcttatgccattcaatcttgtcattccaaccaatgagataacccagccaatcacatccatcaaactggagatagtgacctccaaaagtggtggtcaggcaggggatcagatgtcatggtcggcaagtgggagcctagcagtgacgatccatggtggcaactatccaggggccctccgtcccgtcacactagtagcctacgaaagagtggcaacaggatccgtcgttacggtcgctggggtgagtaacttcgagctgattccaaatcctgaactagcaaagaacctggttacagaatacggccgatttgacccaggagccatgaactacacaaaattgatactgagtgagagggaccgtcttggcatcaagaccgtctggccaacaagggagtacactgattttcgtgagtacttcatggaggtggccgacctcaactctcccctgaagattgcaggagcatttggcttcaaagacataatccgggctataaggaggtaagcttgatctagagcggccgcggggatccagacatgataagatacattgatgagtttggacaaaccacaactagaatgcagtgaaaaaaatgctttatttgtgaaatttgtgatgctattgctttatttgtaaccattataagctgcaataaacaagttaacaacaacaattgcattcattttatgtttcaggttcagggggaggtgtgggaggttttttcggatcctctagagtcgacgaattcgagctcggtacagcttggctgtggaatgtgtgtcagttagggtgtggaaagtccccaggctccccagcaggcagaagtatgcaaagcatgcatctcaattagtcagcaaccaggtgtggaaagtccccaggctccccagcaggcagaagtatgcaaagcatgcatctcaattagtcagcaaccatagtcccgcccctaactccgcccatcccgcccctaactccgcccagttccgcccattctccgccccatggctgactaattttttttatttatgcagaggccgaggccgcctcggcctctgagctattccagaagtagtgaggaggcttttttggaggcctaggcttttgcaaaaagctgcggccgccaccatgggcagcaagcccagcacaagaatcccagcccccctgatgctgatcacccgcatcatgctgatcctgggctgcatcagacccacaagctccctggatggacgccccctggccgctgccggcatcgtggtgaccggcgacaaggccgtgaacgtgtacaccagcagccagaccggcagcatcatcgtgaagctgctgcccaacatgcccagagacaaagaggcctgcgccaaggcccccctggaagcctacaacagaaccctgaccaccctgctgacccccctgggcgacagcatcagaaagatccagggctccgtgagcacaagcggcggaggaaagcagggcagactgatcggcgccgtgatcggcagcgtggccctgggagtggctacagctgcccagattaccgctgcagccgccctgatccaggccaaccagaacgccgccaacatcctgagactgaaagagagcattgccgccaccaacgaggccgtgcacgaagtgaccgacggcctgagccagctgtccgtggccgtgggcaagatgcagcagttcgtgaacgaccagttcaacaacaccgccagagagctggactgcatcaagatcacccagcaggtgggcgtggagctgaacctgtacctgaccgagctgaccacagtgttcggcccccagatcacaagcccagccctgacacagctgaccatccaggccctgtacaacctggctggcggcaacatggactatctgctgacaaagctgggaatcggcaacaaccagctgtccagcctgatcggaagcggcctgatcaccggctaccccatcctgtacgacagccagacacagctgctgggcatccaggtgaacctgcccagcgtgggcaacctgaacaacatgcgcgccacctacctggaaaccctgagcgtgtccaccaccaagggctacgccagcgccctggtgcccaaggtggtgacacaggtgggcagcgtgatcgaggaactggacaccagctactgcatcgagagcgacctggacctgtactgcaccagaatcgtgaccttcccaatgagccccggcatctacagctgcctgagcggcaacaccagcgcctgcatgtacagcaagaccgaaggcgcactgacaacaccctacatggccctgaagggaagcgtgatcgccaactgcaagatcaccacctgcagatgcaccgaccccccaggcatcatcagccagaactacggcgaggccgtgagcctgatcgatcgccattcctgtaacgtgctgtccctggacggcatcacactgagactgagcggcgagttcgatgccacctaccagaagaacatcagcatcctggacagccaggtgatcgtgaccggcaacctggacatcagcaccgagctgggcaacgtgaataacagcatcagcaacgccctggacagactggccgagagcaacagcaagctggaaaaagtgaacgtgcgcctgacatccacttccgctctgatcacctacatcgtgctgaccgtgatcagcctggtgttcggcgccctgagcctggtgctggcctgctacctgatgtacaagcagaaggcccagcagaaaaccctgctgtggctgggcaacaacaccctggaccagatgagagccaccaccagagcctgatgagcggccgcaataaaatatctttattttcattacatctgtgtgttggttttttgtgtgaatcgatagtactaacatacgctctccatcaaaacaaaacgaaacaaaacaaactagcaaaataggctgtccccagtgcaagtgcaggtgccagaacatttctct

SEQ ID NO: 13 - DNA, 3809 bp, artificial sequence
  pFIRESVP2 for vHVT310
  IBDV VP2 (1)..(1362)
  IRES (1363)..(1925)
  NDV-Fopt VIId (1929)..(3590)
  SV40 Poly A (3611)..(3809)
atgacaaacctgcaagatcaaacccaacagattgttccgttcatacggagccttctgatgccaacaaccggaccggcgtccattccggacgacaccctggagaagcacactctcaggtcagagacctcgacctacaatttgactgtgggggacacagggtcagggctaattgtctttttccctggattccctggctcaattgtgggtgctcactacacactgcagagcaatgggaactacaagttcgatcagatgctcctgactgcccagaacctaccggccagctacaactactgcagactagtgagtcggagtctcacagtgaggtcaagcacactccctggtggcgtttatgcactaaacggcaccataaacgccgtgaccttccaaggaagcctgagtgaactgacagatgttagctacaatgggttgatgtctgcaacagccaacatcaacgacaaaattgggaatgtcctggtaggggaaggggtcactgtcctcagcctacccacatcatatgatcttgggtatgtgaggcttggtgaccccattcccgctatagggcttgacccaaaaatggtagctacatgcgacagcagtgacaggcccagagtctacaccataactgcagccgatgattaccaattctcatcacagtaccaaccaggtggggtaacaatcacactgttctcagccaacattgatgctatcacaagcctcagcattgggggagagctcgtgtttcaaacaagcgtccaaggccttgtactgggcgccaccatctaccttataggctttgatgggactgcggtaatcaccagagctgtagccgcagataatgggctgacggccggcaccgacaatcttatgccattcaatcttgtcattccaaccaatgagataacccagccaatcacatccatcaaactggagatagtgacctccaaaagtggtggtcaggcaggggatcagatgtcatggtcggcaagtgggagcctagcagtgacgatccatggtggcaactatccaggggccctccgtcccgtcacactagtagcctacgaaagagtggcaacaggatccgtcgttacggtcgctggggtgagtaacttcgagctgattccaaatcctgaactagcaaagaacctggttacagaatacggccgatttgacccaggagccatgaactacacaaaattgatactgagtgagagggaccgtcttggcatcaagaccgtctggccaacaagggagtacactgattttcgtgagtacttcatggaggtggccgacctcaactctcccctgaagattgcaggagcatttggcttcaaagacataatccgggctataaggaggtaacccccccccctaacgttactggccgaagccgcttggaataaggccggtgtgcgtttgtctatatgttattttccaccatattgccgtcttttggcaatgtgagggcccggaaacctggccctgtcttcttgacgagcattcctaggggtctttcccctctcgccaaaggaatgcaaggtctgttgaatgtcgtgaaggaagcagttcctctggaagcttcttgaagacaaacaacgtctgtagcgaccctttgcaggcagcggaaccccccacctggcgacaggtgcctctgcggccaaaagccacgtgtataagatacacctgcaaaggcggcacaaccccagtgccacgttgtgagttggatagttgtggaaagagtcaaatggctctcctcaagcgtattcaacaaggggctgaaggatgcccagaaggtaccccattgtatgggatctgatctggggcctcggtgcacatgctttacatgtgtttagtcgaggttaaaaaacgtctaggccccccgaaccacggggacgtggttttcctttgaaaaacacgatgataataccatgggcagcaagcccagcacaagaatcccagcccccctgatgctgatcacccgcatcatgctgatcctgggctgcatcagacccacaagctccctggatggacgccccctggccgctgccggcatcgtggtgaccggcgacaaggccgtgaacgtgtacaccagcagccagaccggcagcatcatcgtgaagctgctgcccaacatgcccagagacaaagaggcctgcgccaaggcccccctggaagcctacaacagaaccctgaccaccctgctgacccccctgggcgacagcatcagaaagatccagggctccgtgagcacaagcggcggaggaaagcagggcagactgatcggcgccgtgatcggcagcgtggccctgggagtggctacagctgcccagattaccgctgcagccgccctgatccaggccaaccagaacgccgccaacatcctgagactgaaagagagcattgccgccaccaacgaggccgtgcacgaagtgaccgacggcctgagccagctgtccgtggccgtgggcaagatgcagcagttcgtgaacgaccagttcaacaacaccgccagagagctggactgcatcaagatcacccagcaggtgggcgtggagctgaacctgtacctgaccgagctgaccacagtgttcggcccccagatcacaagcccagccctgacacagctgaccatccaggccctgtacaacctggctggcggcaacatggactatctgctgacaaagctgggaatcggcaacaaccagctgtccagcctgatcggaagcggcctgatcaccggctaccccatcctgtacgacagccagacacagctgctgggcatccaggtgaacctgcccagcgtgggcaacctgaacaacatgcgcgccacctacctggaaaccctgagcgtgtccaccaccaagggctacgccagcgccctggtgcccaaggtggtgacacaggtgggcagcgtgatcgaggaactggacaccagctactgcatcgagagcgacctggacctgtactgcaccagaatcgtgaccttcccaatgagccccggcatctacagctgcctgagcggcaacaccagcgcctgcatgtacagcaagaccgaaggcgcactgacaacaccctacatggccctgaagggaagcgtgatcgccaactgcaagatcaccacctgcagatgcaccgaccccccaggcatcatcagccagaactacggcgaggccgtgagcctgatcgatcgccattcctgtaacgtgctgtccctggacggcatcacactgagactgagcggcgagttcgatgccacctaccagaagaacatcagcatcctggacagccaggtgatcgtgaccggcaacctggacatcagcaccgagctgggcaacgtgaataacagcatcagcaacgccctggacagactggccgagagcaacagcaagctggaaaaagtgaacgtgcgcctgacatccacttccgctctgatcacctacatcgtgctgaccgtgatcagcctggtgttcggcgccctgagcctggtgctggcctgctacctgatgtacaagcagaaggcccagcagaaaaccctgctgtggctgggcaacaacaccctggaccagatgagagccaccaccagagcctgagcttgatctagagcggccgcggggatccagacatgataagatacattgatgagtttggacaaaccacaactagaatgcagtgaaaaaaatgctttatttgtgaaatttgtgatgctattgctttatttgtaaccattataagctgcaataaacaagttaacaacaacaattgcattcattttatgtttcaggttcagggggaggtgtgggaggtttttt

SEQ ID NO: 14 - DNA, 3309 bp, artificial sequence
  pFP2AVP2 for vHVT311
  IBDV VP2 (1)..(1359)
  P2A (1360)..(1425)
  NDV-F wildtype VIId (1426)..(3087)
  SV40 Poly A (3111)..(3309)
atgacaaacctgcaagatcaaacccaacagattgttccgttcatacggagccttctgatgccaacaaccggaccggcgtccattccggacgacaccctggagaagcacactctcaggtcagagacctcgacctacaatttgactgtgggggacacagggtcagggctaattgtctttttccctggattccctggctcaattgtgggtgctcactacacactgcagagcaatgggaactacaagttcgatcagatgctcctgactgcccagaacctaccggccagctacaactactgcagactagtgagtcggagtctcacagtgaggtcaagcacactccctggtggcgtttatgcactaaacggcaccataaacgccgtgaccttccaaggaagcctgagtgaactgacagatgttagctacaatgggttgatgtctgcaacagccaacatcaacgacaaaattgggaatgtcctggtaggggaaggggtcactgtcctcagcctacccacatcatatgatcttgggtatgtgaggcttggtgaccccattcccgctatagggcttgacccaaaaatggtagctacatgcgacagcagtgacaggcccagagtctacaccataactgcagccgatgattaccaattctcatcacagtaccaaccaggtggggtaacaatcacactgttctcagccaacattgatgctatcacaagcctcagcattgggggagagctcgtgtttcaaacaagcgtccaaggccttgtactgggcgccaccatctaccttataggctttgatgggactgcggtaatcaccagagctgtagccgcagataatgggctgacggccggcaccgacaatcttatgccattcaatcttgtcattccaaccaatgagataacccagccaatcacatccatcaaactggagatagtgacctccaaaagtggtggtcaggcaggggatcagatgtcatggtcggcaagtgggagcctagcagtgacgatccatggtggcaactatccaggggccctccgtcccgtcacactagtagcctacgaaagagtggcaacaggatccgtcgttacggtcgctggggtgagtaacttcgagctgattccaaatcctgaactagcaaagaacctggttacagaatacggccgatttgacccaggagccatgaactacacaaaattgatactgagtgagagggaccgtcttggcatcaagaccgtctggccaacaagggagtacactgattttcgtgagtacttcatggaggtggccgacctcaactctcccctgaagattgcaggagcatttggcttcaaagacataatccgggctataaggaggggctccggcgccaccaacttctccctgctcaagcaggccggcgacgtggaggagaaccctggacctatgggctccaaaccttctaccaggatcccagcacctctgatgctgatcacccggattatgctgatattgggctgtatccgtccgacaagctctcttgacggcaggcctcttgcagctgcaggaattgtagtaacaggagataaggcagtcaatgtatacacttcgtctcagacagggtcaatcatagtcaagttgctcccgaatatgcccagggataaggaggcgtgtgcaaaagccccattagaggcatataacagaacactgactactttgctcactcctcttggcgactccatccgcaagatccaagggtctgtgtccacatctggaggaggcaagcaaggccgcctgataggtgctgttattggcagtgtagctcttggggttgcaacagcggcacagataacagcagctgcggccctaatacaagccaaccagaatgccgccaacatcctccggcttaaggagagcattgctgcaaccaatgaagctgtgcatgaagtcaccgacggattatcacaactatcagtggcagttgggaagatgcagcagtttgtcaatgaccagtttaataatacggcgcgagaattggactgtataaaaatcacacaacaggttggtgtagaactcaacctatacctaactgaattgactacagtattcgggccacagatcacctcccctgcattaactcagctgaccatccaggcactttataatttagctggtggcaatatggattacttattaactaagttaggtatagggaacaatcaactcagctcgttaattggtagcggcctgatcactggttaccctatactgtatgactcacagactcaactcttgggcatacaagtgaatttaccctcagtcgggaacttaaataatatgcgtgccacctatttggagaccttatctgtaagtacaaccaaaggatatgcctcagcacttgtcccgaaagtagtgacacaagtcggttccgtgatagaagagcttgacacctcatactgtatagagtccgatctggatttatattgtactagaatagtgacattccccatgtccccaggtatttattcctgtttgagcggcaacacatcagcttgcatgtattcaaagactgaaggcgcactcactacgccgtatatggcccttaaaggctcagttattgccaattgtaaaataacaacatgtagatgtacagaccctcctggtatcatatcgcaaaattatggagaagctgtatccctgatagatagacattcgtgcaatgtcttatcattagacgggataactctaaggctcagtggggaatttgatgcaacttatcaaaagaacatctcaatactagattctcaagtcatcgtgacaggcaatcttgatatatcaactgaacttggaaacgtcaacaattcaatcagcaatgccttggataggttggcagaaagcaacagcaagctagaaaaagtcaatgtcagactaaccagcacatctgctctcattacctatattgttctaactgtcatttctctagttttcggtgcacttagtctggtgttagcgtgttacctgatgtacaaacagaaggcacaacaaaagaccttgctatggcttgggaataataccctcgatcagatgagagccactacaagagcatgataagcttgatctagagcggccgcggggatccagacatgataagatacattgatgagtttggacaaaccacaactagaatgcagtgaaaaaaatgctttatttgtgaaatttgtgatgctattgctttatttgtaaccattataagctgcaataaacaagttaacaacaacaattgcattcattttatgtttcaggttcagggggaggtgtgggaggtttttt

SEQ ID NO: 15 - DNA, 3440 bp, artificial sequence
  pVP2IRESgD for vHVT317
  IBDV VP2 (1)..(1362)
  IRES (1363)..(1925)
  ILTV-gD (1929)..(3233)
  SV40 Poly A (3242)..(3440)
atgacaaacctgcaagatcaaacccaacagattgttccgttcatacggagccttctgatgccaacaaccggaccggcgtccattccggacgacaccctggagaagcacactctcaggtcagagacctcgacctacaatttgactgtgggggacacagggtcagggctaattgtctttttccctggattccctggctcaattgtgggtgctcactacacactgcagagcaatgggaactacaagttcgatcagatgctcctgactgcccagaacctaccggccagctacaactactgcagactagtgagtcggagtctcacagtgaggtcaagcacactccctggtggcgtttatgcactaaacggcaccataaacgccgtgaccttccaaggaagcctgagtgaactgacagatgttagctacaatgggttgatgtctgcaacagccaacatcaacgacaaaattgggaatgtcctggtaggggaaggggtcactgtcctcagcctacccacatcatatgatcttgggtatgtgaggcttggtgaccccattcccgctatagggcttgacccaaaaatggtagctacatgcgacagcagtgacaggcccagagtctacaccataactgcagccgatgattaccaattctcatcacagtaccaaccaggtggggtaacaatcacactgttctcagccaacattgatgctatcacaagcctcagcattgggggagagctcgtgtttcaaacaagcgtccaaggccttgtactgggcgccaccatctaccttataggctttgatgggactgcggtaatcaccagagctgtagccgcagataatgggctgacggccggcaccgacaatcttatgccattcaatcttgtcattccaaccaatgagataacccagccaatcacatccatcaaactggagatagtgacctccaaaagtggtggtcaggcaggggatcagatgtcatggtcggcaagtgggagcctagcagtgacgatccatggtggcaactatccaggggccctccgtcccgtcacactagtagcctacgaaagagtggcaacaggatccgtcgttacggtcgctggggtgagtaacttcgagctgattccaaatcctgaactagcaaagaacctggttacagaatacggccgatttgacccaggagccatgaactacacaaaattgatactgagtgagagggaccgtcttggcatcaagaccgtctggccaacaagggagtacactgattttcgtgagtacttcatggaggtggccgacctcaactctcccctgaagattgcaggagcatttggcttcaaagacataatccgggctataaggaggtaacccccccccctaacgttactggccgaagccgcttggaataaggccggtgtgcgtttgtctatatgttattttccaccatattgccgtcttttggcaatgtgagggcccggaaacctggccctgtcttcttgacgagcattcctaggggtctttcccctctcgccaaaggaatgcaaggtctgttgaatgtcgtgaaggaagcagttcctctggaagcttcttgaagacaaacaacgtctgtagcgaccctttgcaggcagcggaaccccccacctggcgacaggtgcctctgcggccaaaagccacgtgtataagatacacctgcaaaggcggcacaaccccagtgccacgttgtgagttggatagttgtggaaagagtcaaatggctctcctcaagcgtattcaacaaggggctgaaggatgcccagaaggtaccccattgtatgggatctgatctggggcctcggtgcacatgctttacatgtgtttagtcgaggttaaaaaacgtctaggccccccgaaccacggggacgtggttttcctttgaaaaacacgatgataataccatgcaccgtcctcatctcagacggcactcgcgttactacgcgaaaggagaggtgcttaacaaacacatggattgcggtggaaaacggtgctgctcaggcgcagctgtattcactcttttctggacttgtgtcaggattatgcgggagcatatctgctttgtacgcaacgctatggaccgccatttatttttgaggaatgctttttggactatcgtactgctttcttccttcgctagccagagcaccgccgccgtcacgtacgactacattttaggccgtcgcgcgctcgacgcgctaaccataccggcggttggcccgtataacagatacctcactagggtatcaagaggctgcgacgttgtcgagctcaacccgatttctaacgtggacgacatgatatcggcggccaaagaaaaagagaaggggggccctttcgaggcctccgtcgtctggttctacgtgattaagggcgacgacggcgaggacaagtactgtccaatctatagaaaagagtacagggaatgtggcgacgtacaactgctatctgaatgcgccgttcaatctgcacagatgtgggcagtggactatgttcctagcacccttgtatcgcgaaatggcgcgggactgactatattctcccccactgctgcgctctctggccaatacttgctgaccctgaaaatcgggagatttgcgcaaacagctctcgtaactctagaagttaacgatcgctgtttaaagatcgggtcgcagcttaactttttaccgtcgaaatgctggacaacagaacagtatcagactggatttcaaggcgaacacctttatccgatcgcagacaccaatacacgacacgcggacgacgtatatcggggatacgaagatattctgcagcgctggaataatttgctgaggaaaaagaatcctagcgcgccagaccctcgtccagatagcgtcccgcaagaaattcccgctgtaaccaagaaagcggaagggcgcaccccggacgcagaaagcagcgaaaagaaggcccctccagaagactcggaggacgacatgcaggcagaggcttctggagaaaatcctgccgccctccccgaagacgacgaagtccccgaggacaccgagcacgatgatccaaactcggatcctgactattacaatgacatgcccgccgtgatcccggtggaggagactactaaaagttctaatgccgtctccatgcccatattcgcggcgttcgtagcctgcgcggtcgcgctcgtggggctactggtttggagcatcgtaaaatgcgcgcgtagctaagcggccgcggggatccagacatgataagatacattgatgagtttggacaaaccacaactagaatgcagtgaaaaaaatgctttatttgtgaaatttgtgatgctattgctttatttgtaaccattataagctgcaataaacaagttaacaacaacaattgcattcattttatgtttcaggttcagggggaggtgtgggaggtttttt

SEQ ID NO: 16 - DNA, 1302 bp, artificial sequence
  Polynucleotide encoding ILTV gD
atgcaccgtcctcatctcagacggcactcgcgttactacgcgaaaggagaggtgcttaacaaacacatggattgcggtggaaaacggtgctgctcaggcgcagctgtattcactcttttctggacttgtgtcaggattatgcgggagcatatctgctttgtacgcaacgctatggaccgccatttatttttgaggaatgctttttggactatcgtactgctttcttccttcgctagccagagcaccgccgccgtcacgtacgactacattttaggccgtcgcgcgctcgacgcgctaaccataccggcggttggcccgtataacagatacctcactagggtatcaagaggctgcgacgttgtcgagctcaacccgatttctaacgtggacgacatgatatcggcggccaaagaaaaagagaaggggggccctttcgaggcctccgtcgtctggttctacgtgattaagggcgacgacggcgaggacaagtactgtccaatctatagaaaagagtacagggaatgtggcgacgtacaactgctatctgaatgcgccgttcaatctgcacagatgtgggcagtggactatgttcctagcacccttgtatcgcgaaatggcgcgggactgactatattctcccccactgctgcgctctctggccaatacttgctgaccctgaaaatcgggagatttgcgcaaacagctctcgtaactctagaagttaacgatcgctgtttaaagatcgggtcgcagcttaactttttaccgtcgaaatgctggacaacagaacagtatcagactggatttcaaggcgaacacctttatccgatcgcagacaccaatacacgacacgcggacgacgtatatcggggatacgaagatattctgcagcgctggaataatttgctgaggaaaaagaatcctagcgcgccagaccctcgtccagatagcgtcccgcaagaaattcccgctgtaaccaagaaagcggaagggcgcaccccggacgcagaaagcagcgaaaagaaggcccctccagaagactcggaggacgacatgcaggcagaggcttctggagaaaatcctgccgccctccccgaagacgacgaagtccccgaggacaccgagcacgatgatccaaactcggatcctgactattacaatgacatgcccgccgtgatcccggtggaggagactactaaaagttctaatgccgtctccatgcccatattcgcggcgttcgtagcctgcgcggtcgcgctcgtggggctactggtttggagcatcgtaaaatgcgcgcgtagc

SEQ ID NO: 17 - protein, 434 aa, artificial sequence
  ILTV gD protein
MHRPHLRRHSRYYAKGEVLNKHMDCGGKRCCSGAAVFTLFWTCVRIMREHICFVRNAMDRHLFLRNAFWTIVLLSSFASQSTAAVTYDYILGRRALDALTIPAVGPYNRYLTRVSRGCDVVELNPISNVDDMISAAKEKEKGGPFEASVVWFYVIKGDDGEDKYCPIYRKEYRECGDVQLLSECAVQSAQMWAVDYVPSTLVSRNGAGLTIFSPTAALSGQYLLTLKIGRFAQTALVTLEVNDRCLKIGSQLNFLPSKCWTTEQYQTGFQGEHLYPIADTNTRHADDVYRGYEDILQRWNNLLRKKNPSAPDPRPDSVPQEIPAVTKKAEGRTPDAESSEKKAPPEDSEDDMQAEASGENPAALPEDDEVPEDTEHDDPNSDPDYYNDMPAVIPVEETTKSSNAVSMPIFAAFVACAVALVGLLVWSIVKCARS

SEQ ID NO: 18 - DNA, 3804 bp, artificial sequence
  pFwtSV40VP2 for vHFT313
  VP2 (1)..(1362)
  SV40 Poly A (1383)..(1594)
  SV40 Promoter (1624)..(1968)
  NDV-Fwt VIId (1981)..(3642)
  Synthetic Poly A (3651)..(3804)
atgacaaacctgcaagatcaaacccaacagattgttccgttcatacggagccttctgatgccaacaaccggaccggcgtccattccggacgacaccctggagaagcacactctcaggtcagagacctcgacctacaatttgactgtgggggacacagggtcagggctaattgtctttttccctggattccctggctcaattgtgggtgctcactacacactgcagagcaatgggaactacaagttcgatcagatgctcctgactgcccagaacctaccggccagctacaactactgcagactagtgagtcggagtctcacagtgaggtcaagcacactccctggtggcgtttatgcactaaacggcaccataaacgccgtgaccttccaaggaagcctgagtgaactgacagatgttagctacaatgggttgatgtctgcaacagccaacatcaacgacaaaattgggaatgtcctggtaggggaaggggtcactgtcctcagcctacccacatcatatgatcttgggtatgtgaggcttggtgaccccattcccgctatagggcttgacccaaaaatggtagctacatgcgacagcagtgacaggcccagagtctacaccataactgcagccgatgattaccaattctcatcacagtaccaaccaggtggggtaacaatcacactgttctcagccaacattgatgctatcacaagcctcagcattgggggagagctcgtgtttcaaacaagcgtccaaggccttgtactgggcgccaccatctaccttataggctttgatgggactgcggtaatcaccagagctgtagccgcagataatgggctgacggccggcaccgacaatcttatgccattcaatcttgtcattccaaccaatgagataacccagccaatcacatccatcaaactggagatagtgacctccaaaagtggtggtcaggcaggggatcagatgtcatggtcggcaagtgggagcctagcagtgacgatccatggtggcaactatccaggggccctccgtcccgtcacactagtagcctacgaaagagtggcaacaggatccgtcgttacggtcgctggggtgagtaacttcgagctgattccaaatcctgaactagcaaagaacctggttacagaatacggccgatttgacccaggagccatgaactacacaaaattgatactgagtgagagggaccgtcttggcatcaagaccgtctggccaacaagggagtacactgattttcgtgagtacttcatggaggtggccgacctcaactctcccctgaagattgcaggagcatttggcttcaaagacataatccgggctataaggaggtaagcttgatctagagcggccgcggggatccagacatgataagatacattgatgagtttggacaaaccacaactagaatgcagtgaaaaaaatgctttatttgtgaaatttgtgatgctattgctttatttgtaaccattataagctgcaataaacaagttaacaacaacaattgcattcattttatgtttcaggttcagggggaggtgtgggaggttttttcggatcctctagagtcgacgaattcgagctcggtacagcttggctgtggaatgtgtgtcagttagggtgtggaaagtccccaggctccccagcaggcagaagtatgcaaagcatgcatctcaattagtcagcaaccaggtgtggaaagtccccaggctccccagcaggcagaagtatgcaaagcatgcatctcaattagtcagcaaccatagtcccgcccctaactccgcccatcccgcccctaactccgcccagttccgcccattctccgccccatggctgactaattttttttatttatgcagaggccgaggccgcctcggcctctgagctattccagaagtagtgaggaggcttttttggaggcctaggcttttgcaaaaagctgcggccgccaccatgggctccaaaccttctaccaggatcccagcacctctgatgctgatcacccggattatgctgatattgggctgtatccgtccgacaagctctcttgacggcaggcctcttgcagctgcaggaattgtagtaacaggagataaggcagtcaatgtatacacttcgtctcagacagggtcaatcatagtcaagttgctcccgaatatgcccagggataaggaggcgtgtgcaaaagccccattagaggcatataacagaacactgactactttgctcactcctcttggcgactccatccgcaagatccaagggtctgtgtccacatctggaggaggcaagcaaggccgcctgataggtgctgttattggcagtgtagctcttggggttgcaacagcggcacagataacagcagctgcggccctaatacaagccaaccagaatgccgccaacatcctccggcttaaggagagcattgctgcaaccaatgaagctgtgcatgaagtcaccgacggattatcacaactatcagtggcagttgggaagatgcagcagtttgtcaatgaccagtttaataatacggcgcgagaattggactgtataaaaatcacacaacaggttggtgtagaactcaacctatacctaactgaattgactacagtattcgggccacagatcacctcccctgcattaactcagctgaccatccaggcactttataatttagctggtggcaatatggattacttattaactaagttaggtatagggaacaatcaactcagctcgttaattggtagcggcctgatcactggttaccctatactgtatgactcacagactcaactcttgggcatacaagtgaatttaccctcagtcgggaacttaaataatatgcgtgccacctatttggagaccttatctgtaagtacaaccaaaggatatgcctcagcacttgtcccgaaagtagtgacacaagtcggttccgtgatagaagagcttgacacctcatactgtatagagtccgatctggatttatattgtactagaatagtgacattccccatgtccccaggtatttattcctgtttgagcggcaacacatcagcttgcatgtattcaaagactgaaggcgcactcactacgccgtatatggcccttaaaggctcagttattgccaattgtaaaataacaacatgtagatgtacagaccctcctggtatcatatcgcaaaattatggagaagctgtatccctgatagatagacattcgtgcaatgtcttatcattagacgggataactctaaggctcagtggggaatttgatgcaacttatcaaaagaacatctcaatactagattctcaagtcatcgtgacaggcaatcttgatatatcaactgaacttggaaacgtcaacaattcaatcagcaatgccttggataggttggcagaaagcaacagcaagctagaaaaagtcaatgtcagactaaccagcacatctgctctcattacctatattgttctaactgtcatttctctagttttcggtgcacttagtctggtgttagcgtgttacctgatgtacaaacagaaggcacaacaaaagaccttgctatggcttgggaataataccctcgatcagatgagagccactacaagagcatgagcggccgcaataaaatatctttattttcattacatctgtgtgttggttttttgtgtgaatcgatagtactaacatacgctctccatcaaaacaaaacgaaacaaaacaaactagcaaaataggctgtccccagtgcaagtgcaggtgccagaacatttctct

SEQ ID NO: 19 - DNA, 3797 bp, artificial sequence
  pVP2IRESFwt for vHVT316
  VP2 (1)..(1362)
  IRES (1363)..(1925)
  NDV-Fwt VIId (1929)..(3590)
  SV40 Poly A (3599)..(3797)
atgacaaacctgcaagatcaaacccaacagattgttccgttcatacggagccttctgatgccaacaaccggaccggcgtccattccggacgacaccctggagaagcacactctcaggtcagagacctcgacctacaatttgactgtgggggacacagggtcagggctaattgtctttttccctggattccctggctcaattgtgggtgctcactacacactgcagagcaatgggaactacaagttcgatcagatgctcctgactgcccagaacctaccggccagctacaactactgcagactagtgagtcggagtctcacagtgaggtcaagcacactccctggtggcgtttatgcactaaacggcaccataaacgccgtgaccttccaaggaagcctgagtgaactgacagatgttagctacaatgggttgatgtctgcaacagccaacatcaacgacaaaattgggaatgtcctggtaggggaaggggtcactgtcctcagcctacccacatcatatgatcttgggtatgtgaggcttggtgaccccattcccgctatagggcttgacccaaaaatggtagctacatgcgacagcagtgacaggcccagagtctacaccataactgcagccgatgattaccaattctcatcacagtaccaaccaggtggggtaacaatcacactgttctcagccaacattgatgctatcacaagcctcagcattgggggagagctcgtgtttcaaacaagcgtccaaggccttgtactgggcgccaccatctaccttataggctttgatgggactgcggtaatcaccagagctgtagccgcagataatgggctgacggccggcaccgacaatcttatgccattcaatcttgtcattccaaccaatgagataacccagccaatcacatccatcaaactggagatagtgacctccaaaagtggtggtcaggcaggggatcagatgtcatggtcggcaagtgggagcctagcagtgacgatccatggtggcaactatccaggggccctccgtcccgtcacactagtagcctacgaaagagtggcaacaggatccgtcgttacggtcgctggggtgagtaacttcgagctgattccaaatcctgaactagcaaagaacctggttacagaatacggccgatttgacccaggagccatgaactacacaaaattgatactgagtgagagggaccgtcttggcatcaagaccgtctggccaacaagggagtacactgattttcgtgagtacttcatggaggtggccgacctcaactctcccctgaagattgcaggagcatttggcttcaaagacataatccgggctataaggaggtaacccccccccctaacgttactggccgaagccgcttggaataaggccggtgtgcgtttgtctatatgttattttccaccatattgccgtcttttggcaatgtgagggcccggaaacctggccctgtcttcttgacgagcattcctaggggtctttcccctctcgccaaaggaatgcaaggtctgttgaatgtcgtgaaggaagcagttcctctggaagcttcttgaagacaaacaacgtctgtagcgaccctttgcaggcagcggaaccccccacctggcgacaggtgcctctgcggccaaaagccacgtgtataagatacacctgcaaaggcggcacaaccccagtgccacgttgtgagttggatagttgtggaaagagtcaaatggctctcctcaagcgtattcaacaaggggctgaaggatgcccagaaggtaccccattgtatgggatctgatctggggcctcggtgcacatgctttacatgtgtttagtcgaggttaaaaaacgtctaggccccccgaaccacggggacgtggttttcctttgaaaaacacgatgataataccatgggctccaaaccttctaccaggatcccagcacctctgatgctgatcacccggattatgctgatattgggctgtatccgtccgacaagctctcttgacggcaggcctcttgcagctgcaggaattgtagtaacaggagataaggcagtcaatgtatacacttcgtctcagacagggtcaatcatagtcaagttgctcccgaatatgcccagggataaggaggcgtgtgcaaaagccccattagaggcatataacagaacactgactactttgctcactcctcttggcgactccatccgcaagatccaagggtctgtgtccacatctggaggaggcaagcaaggccgcctgataggtgctgttattggcagtgtagctcttggggttgcaacagcggcacagataacagcagctgcggccctaatacaagccaaccagaatgccgccaacatcctccggcttaaggagagcattgctgcaaccaatgaagctgtgcatgaagtcaccgacggattatcacaactatcagtggcagttgggaagatgcagcagtttgtcaatgaccagtttaataatacggcgcgagaattggactgtataaaaatcacacaacaggttggtgtagaactcaacctatacctaactgaattgactacagtattcgggccacagatcacctcccctgcattaactcagctgaccatccaggcactttataatttagctggtggcaatatggattacttattaactaagttaggtatagggaacaatcaactcagctcgttaattggtagcggcctgatcactggttaccctatactgtatgactcacagactcaactcttgggcatacaagtgaatttaccctcagtcgggaacttaaataatatgcgtgccacctatttggagaccttatctgtaagtacaaccaaaggatatgcctcagcacttgtcccgaaagtagtgacacaagtcggttccgtgatagaagagcttgacacctcatactgtatagagtccgatctggatttatattgtactagaatagtgacattccccatgtccccaggtatttattcctgtttgagcggcaacacatcagcttgcatgtattcaaagactgaaggcgcactcactacgccgtatatggcccttaaaggctcagttattgccaattgtaaaataacaacatgtagatgtacagaccctcctggtatcatatcgcaaaattatggagaagctgtatccctgatagatagacattcgtgcaatgtcttatcattagacgggataactctaaggctcagtggggaatttgatgcaacttatcaaaagaacatctcaatactagattctcaagtcatcgtgacaggcaatcttgatatatcaactgaacttggaaacgtcaacaattcaatcagcaatgccttggataggttggcagaaagcaacagcaagctagaaaaagtcaatgtcagactaaccagcacatctgctctcattacctatattgttctaactgtcatttctctagttttcggtgcacttagtctggtgttagcgtgttacctgatgtacaaacagaaggcacaacaaaagaccttgctatggcttgggaataataccctcgatcagatgagagccactacaagagcatgaggcgcgccggggatccagacatgataagatacattgatgagtttggacaaaccacaactagaatgcagtgaaaaaaatgctttatttgtgaaatttgtgatgctattgctttatttgtaaccattataagctgcaataaacaagttaacaacaacaattgcattcattttatgtttcaggttcagggggaggtgtgggaggtttttt

SEQ ID NO: 20 - DNA, 1834 bp, artificial sequence
  HVT US2SVgDwtsyn for vHVT407
  SV40 Promoter (1)..(345)
  ILTV gDwt (362)..(1666)
  synthetic poly A (1681)..(1834)
gctgtggaatgtgtgtcagttagggtgtggaaagtccccaggctccccagcaggcagaagtatgcaaagcatgcatctcaattagtcagcaaccaggtgtggaaagtccccaggctccccagcaggcagaagtatgcaaagcatgcatctcaattagtcagcaaccatagtcccgcccctaactccgcccatcccgcccctaactccgcccagttccgcccattctccgccccatggctgactaattttttttatttatgcagaggccgaggccgcctcggcctctgagctattccagaagtagtgaggaggcttttttggaggcctaggcttttgcaaaaagctgcggccggccgccaccatgcaccgtcctcatctcagacggcactcgcgttactacgcgaaaggagaggtgcttaacaaacacatggattgcggtggaaaacggtgctgctcaggcgcagctgtattcactcttttctggacttgtgtcaggattatgcgggagcatatctgctttgtacgcaacgctatggaccgccatttatttttgaggaatgctttttggactatcgtactgctttcttccttcgctagccagagcaccgccgccgtcacgtacgactacattttaggccgtcgcgcgctcgacgcgctaaccataccggcggttggcccgtataacagatacctcactagggtatcaagaggctgcgacgttgtcgagctcaacccgatttctaacgtggacgacatgatatcggcggccaaagaaaaagagaaggggggccctttcgaggcctccgtcgtctggttctacgtgattaagggcgacgacggcgaggacaagtactgtccaatctatagaaaagagtacagggaatgtggcgacgtacaactgctatctgaatgcgccgttcaatctgcacagatgtgggcagtggactatgttcctagcacccttgtatcgcgaaatggcgcgggactgactatattctcccccactgctgcgctctctggccaatacttgctgaccctgaaaatcgggagatttgcgcaaacagctctcgtaactctagaagttaacgatcgctgtttaaagatcgggtcgcagcttaactttttaccgtcgaaatgctggacaacagaacagtatcagactggatttcaaggcgaacacctttatccgatcgcagacaccaatacacgacacgcggacgacgtatatcggggatacgaagatattctgcagcgctggaataatttgctgaggaaaaagaatcctagcgcgccagaccctcgtccagatagcgtcccgcaagaaattcccgctgtaaccaagaaagcggaagggcgcaccccggacgcagaaagcagcgaaaagaaggcccctccagaagactcggaggacgacatgcaggcagaggcttctggagaaaatcctgccgccctccccgaagacgacgaagtccccgaggacaccgagcacgatgatccaaactcggatcctgactattacaatgacatgcccgccgtgatcccggtggaggagactactaaaagttctaatgccgtctccatgcccatattcgcggcgttcgtagcctgcgcggtcgcgctcgtggggctactggtttggagcatcgtaaaatgcgcgcgtagctaatcgagcctagaggcaataaaatatctttattttcattacatctgtgtgttggttttttgtgtgaatcgatagtactaacatacgctctccatcaaaacaaaacgaaacaaaacaaactagcaaaataggctgtccccagtgcaagtgcaggtgccagaacatttctct

SEQ ID NO: 21 - DNA, 1659 bp, artificial sequence
  Polynucleotide encoding NDV-F of genotype V, codon-optimized in pHVTIG1gDCaFopt (vHVT308)
atgggcagcaagcccagcacctggatcagcgtgaccctgatgctgatcaccagaaccatgctgatcctgagctgcatctgccccacaagcagcctggacggcagacccctggccgctgccggcatcgtggtgaccggcgacaaggccgtgaacatctacaccagcagccagaccggcagcatcatcatcaagctgctgcccaacatgcccaaggacaaagaggcctgcgccaaggcccccctggaagcctacaacagaaccctgaccaccctgctgacccccctgggcgacagcatcagaagaatccagggcagcgccaccacaagcggcggaggaaagcagggcagactggtgggcgctatcatcgggagcgtggccctgggcgtggccacagctgcccagattaccgctgcagccgccctgattcaggccaatcagaacgccgccaacatcctgagactgaaagagagcattgccgccaccaacgacgccgtgcacgaagtgacaaacggactgtcccagctggctgtcgctgtcggcaagatgcagcagttcgtgaacaaccagttcaacaacaccgccagagagctggactgcatcaagatcgcccagcaggtgggcgtggagctgaacctgtacctgaccgagctgaccacagtgttcggcccccagatcacaagccccgctctgacccagctgacaatccaggccctgtacaacctggctggcggcaacatggactatctgctgactaagctgggagtgggcaacaaccagctgtccagcctgatcgggtccgggctgatcacaggcaaccccatcctgtacgacagccagacacagctgctgggcatccagatcaacctgccatccgtgggaagcctgaacaacatgagagccacctacctggaaaccctgagcgtgtccaccaccaagggcttcgccagcgccctggtgcccaaggtggtgacacaggtgggcagcgtgatcgaggaactggacaccagctactgcatcgagagcgacatcgacctgtactgcaccagagtggtgaccttcccaatgagccccggcatctacagctgcctgagcggcaacaccagcgcctgcatgtacagcaagaccgaaggagcactgacaacaccctacatggccctgaagggaagcgtgatcgccaactgcaagatgaccacctgcagatgcgccgaccccccaggcatcatcagccagaactacggcgaggccgtgagcctgatcgacaaacattcctgtagcgtgctgtccctggatggcatcacactgagactgagcggcgagttcgacgccacctaccagaagaacatcagcatcctggacagccaggtgatcgtgaccggcaacctggacatcagcaccgagctgggcaacgtgaacaacagcatcagcagcaccctggacaagctggccgagtccaacaacaagctgaacaaagtgaacgtgaacctgaccagcacaagcgccctgatcacctacatcgtgctggccatcgtgtccctggccttcggcgtgatcagcctggtgctggcctgctacctgatgtacaagcagagagcccagcagaaaaccctgctgtggctgggcaataacaccctggaccagatgagggccaccaccagaacc

SEQ ID NO: 22 - protein, 553 aa, artificial sequence
  NDV-F of genotype V (vHVT308)
MGSKPSTWISVTLMLITRTMLILSCICPTSSLDGRPLAAAGIVVTGDKAVNIYTSSQTGSIIIKLLPNMPKDKEACAKAPLEAYNRTLTTLLTPLGDSIRRIQGSATTSGGGKQGRLVGAIIGSVALGVATAAQITAAAALIQANQNAANILRLKESIAATNDAVHEVTNGLSQLAVAVGKMQQFVNNQFNNTARELDCIKIAQQVGVELNLYLTELTTVFGPQITSPALTQLTIQALYNLAGGNMDYLLTKLGVGNNQLSSLIGSGLITGNPILYDSQTQLLGIQINLPSVGSLNNMRATYLETLSVSTTKGFASALVPKVVTQVGSVIEELDTSYCIESDIDLYCTRVVTFPMSPGIYSCLSGNTSACMYSKTEGALTTPYMALKGSVIANCKMTTCRCADPPGIISQNYGEAVSLIDKHSCSVLSLDGITLRLSGEFDATYQKNISILDSQVIVTGNLDISTELGNVNNSISSTLDKLAESNNKLNKVNVNLTSTSALITYIVLAIVSLAFGVISLVLACYLMYKQRAQQKTLLWLGNNTLDQMRATTRT

SEQ ID NO: 23 - DNA, 476 bp, artificial sequence
  HHV3gB promoter (reverse direction)
cccgggttatatcttctgattgtgtgggctctacttgtaaactctcaaaaaacgagcttggagagaccgacacaaccgccgtaacaaacaaagaaaatatgcataaaaagcataaccacacccccgtaacggatgttatgaaaacgccgggtccgttgaatccggagccagccgctgcattagggtgtatagaagagaaaaaacgtctgaatcgtagattacgacggtattctggtcgatccctgtttctccactttgaataatagccacaaggggacatgtttcttcgtacgttaaataaatgccgtctaagggtccgtgggaactgcctatacctttaggttgagacgtgcacccgcgtggatccttacctagacggtcaacgcgacataaccgcacctccccacaatggaaaacagaggtgaatagtgtggttgcaaacacaagctccctaatatatttccaggcaagtctct

SEQ ID NO: 24 - DNA, 476 bp, artificial sequence
  HHV3gB promoter
agagacttgcctggaaatatattagggagcttgtgtttgcaaccacactattcacctctgttttccattgtggggaggtgcggttatgtcgcgttgaccgtctaggtaaggatccacgcgggtgcacgtctcaacctaaaggtataggcagttcccacggacccttagacggcatttatttaacgtacgaagaaacatgtccccttgtggctattattcaaagtggagaaacagggatcgaccagaataccgtcgtaatctacgattcagacgttttttctcttctatacaccctaatgcagcggctggctccggattcaacggacccggcgttttcataacatccgttacgggggtgtggttatgctttttatgcatattttctttgtttgttacggcggttgtgtcggtctctccaagctcgttttttgagagtttacaagtagagcccacacaatcagaagatataacccggg

SEQ ID NO: 25 - DNA, 4347 bp, artificial sequence
  Plasmid pHVTIG1gDCaFopt for vHVT308
  SV40 Poly A in reverse direction (1)..(199)
  ILTgD  in reverse direction (318)..(1622)
  HHV3gB promoter  in reverse direction (1635)..(2110)
  SV40 promoter (2129)..(2496)
  NDV-F-CA02 (2515)..(4179)
  Syn Poly A (4194)..(4347)
aaaaaacctcccacacctccccctgaacctgaaacataaaatgaatgcaattgttgttgttaacttgtttattgcagcttataatggttacaaataaagcaatagcatcacaaatttcacaaataaagcatttttttcactgcattctagttgtggtttgtccaaactcatcaatgtatcttatcatgtctggatccccgcggcctatgcgcttttcgaacgtcccaatgaataggcattggtatgctattccatgtgatttatattatgagcgtgaggcgtggcatgtaggaagaaaccacctattctaggctcgattagctacgcgcgcattttacgatgctccaaaccagtagccccacgagcgcgaccgcgcaggctacgaacgccgcgaatatgggcatggagacggcattagaacttttagtagtctcctccaccgggatcacggcgggcatgtcattgtaatagtcaggatccgagtttggatcatcgtgctcggtgtcctcggggacttcgtcgtcttcggggagggcggcaggattttctccagaagcctctgcctgcatgtcgtcctccgagtcttctggaggggccttcttttcgctgctttctgcgtccggggtgcgcccttccgctttcttggttacagcgggaatttcttgcgggacgctatctggacgagggtctggcgcgctaggattctttttcctcagcaaattattccagcgctgcagaatatcttcgtatccccgatatacgtcgtccgcgtgtcgtgtattggtgtctgcgatcggataaaggtgttcgccttgaaatccagtctgatactgttctgttgtccagcatttcgacggtaaaaagttaagctgcgacccgatctttaaacagcgatcgttaacttctagagttacgagagctgtttgcgcaaatctcccgattttcagggtcagcaagtattggccagagagcgcagcagtgggggagaatatagtcagtcccgcgccatttcgcgatacaagggtgctaggaacatagtccactgcccacatctgtgcagattgaacggcgcattcagatagcagttgtacgtcgccacattccctgtactcttttctatagattggacagtacttgtcctcgccgtcgtcgcccttaatcacgtagaaccagacgacggaggcctcgaaagggccccccttctctttttctttggccgccgatatcatgtcgtccacgttagaaatcgggttgagctcgacaacgtcgcagcctcttgataccctagtgaggtatctgttatacgggccaaccgccggtatggttagcgcgtcgagcgcgcgacggcctaaaatgtagtcgtacgtgacggcggcggtgctctggctagcgaaggaagaaagcagtacgatagtccaaaaagcattcctcaaaaataaatggcggtccatagcgttgcgtacaaagcagatatgctcccgcataatcctgacacaagtccagaaaagagtgaatacagctgcgcctgagcagcaccgttttccaccgcaatccatgtgtttgttaagcacctctcctttcgcgtagtaacgcgagtgccgtctgagatgaggacggtgcatggtggcggccgccccgggttatatcttctgattgtgtgggctctacttgtaaactctcaaaaaacgagcttggagagaccgacacaaccgccgtaacaaacaaagaaaatatgcataaaaagcataaccacacccccgtaacggatgttatgaaaacgccgggtccgttgaatccggagccagccgctgcattagggtgtatagaagagaaaaaacgtctgaatcgtagattacgacggtattctggtcgatccctgtttctccactttgaataatagccacaaggggacatgtttcttcgtacgttaaataaatgccgtctaagggtccgtgggaactgcctatacctttaggttgagacgtgcacccgcgtggatccttacctagacggtcaacgcgacataaccgcacctccccacaatggaaaacagaggtgaatagtgtggttgcaaacacaagctccctaatatatttccaggcaagtctctgaattaattccctcgacccaattcgagctcggtacagcttggctgtggaatgtgtgtcagttagggtgtggaaagtccccaggctccccagcaggcagaagtatgcaaagcatgcatctcaattagtcagcaaccaggtgtggaaagtccccaggctccccagcaggcagaagtatgcaaagcatgcatctcaattagtcagcaaccatagtcccgcccctaactccgcccatcccgcccctaactccgcccagttccgcccattctccgccccatggctgactaattttttttatttatgcagaggccgaggccgcctcggcctctgagctattccagaagtagtgaggaggcttttttggaggcctaggcttttgcaaaaagctcccggggcggccgccaccatgggcagcaagcccagcacctggatcagcgtgaccctgatgctgatcaccagaaccatgctgatcctgagctgcatctgccccacaagcagcctggacggcagacccctggccgctgccggcatcgtggtgaccggcgacaaggccgtgaacatctacaccagcagccagaccggcagcatcatcatcaagctgctgcccaacatgcccaaggacaaagaggcctgcgccaaggcccccctggaagcctacaacagaaccctgaccaccctgctgacccccctgggcgacagcatcagaagaatccagggcagcgccaccacaagcggcggaggaaagcagggcagactggtgggcgctatcatcgggagcgtggccctgggcgtggccacagctgcccagattaccgctgcagccgccctgattcaggccaatcagaacgccgccaacatcctgagactgaaagagagcattgccgccaccaacgacgccgtgcacgaagtgacaaacggactgtcccagctggctgtcgctgtcggcaagatgcagcagttcgtgaacaaccagttcaacaacaccgccagagagctggactgcatcaagatcgcccagcaggtgggcgtggagctgaacctgtacctgaccgagctgaccacagtgttcggcccccagatcacaagccccgctctgacccagctgacaatccaggccctgtacaacctggctggcggcaacatggactatctgctgactaagctgggagtgggcaacaaccagctgtccagcctgatcgggtccgggctgatcacaggcaaccccatcctgtacgacagccagacacagctgctgggcatccagatcaacctgccatccgtgggaagcctgaacaacatgagagccacctacctggaaaccctgagcgtgtccaccaccaagggcttcgccagcgccctggtgcccaaggtggtgacacaggtgggcagcgtgatcgaggaactggacaccagctactgcatcgagagcgacatcgacctgtactgcaccagagtggtgaccttcccaatgagccccggcatctacagctgcctgagcggcaacaccagcgcctgcatgtacagcaagaccgaaggagcactgacaacaccctacatggccctgaagggaagcgtgatcgccaactgcaagatgaccacctgcagatgcgccgaccccccaggcatcatcagccagaactacggcgaggccgtgagcctgatcgacaaacattcctgtagcgtgctgtccctggatggcatcacactgagactgagcggcgagttcgacgccacctaccagaagaacatcagcatcctggacagccaggtgatcgtgaccggcaacctggacatcagcaccgagctgggcaacgtgaacaacagcatcagcagcaccctggacaagctggccgagtccaacaacaagctgaacaaagtgaacgtgaacctgaccagcacaagcgccctgatcacctacatcgtgctggccatcgtgtccctggccttcggcgtgatcagcctggtgctggcctgctacctgatgtacaagcagagagcccagcagaaaaccctgctgtggctgggcaataacaccctggaccagatgagggccaccaccagaacctgatgagcggccgcgatatcaataaaatatctttattttcattacatctgtgtgttggttttttgtgtgaatcgatagtactaacatacgctctccatcaaaacaaaacgaaacaaaacaaactagcaaaataggctgtccccagtgcaagtgcaggtgccagaacatttctct

SEQ ID NO: 26 - DNA, 5149 bp, artificial sequence
  Plasmid pFwtIRESgD for vHVT322
  mCMV promoter (1)..(1391)
  NDV-Fwt VIId (1400)..(3061)
  IRES (3072)..(3634)
  ILTgD (3638)..(4942)
  SV40 Poly A (4951)..(5149)
aactccgcccgttttatgactagaaccaatagtttttaatgccaaatgcactgaaatcccctaatttgcaaagccaaacgccccctatgtgagtaatacggggactttttacccaatttcccacgcggaaagccccctaatacactcatatggcatatgaatcagcacggtcatgcactctaatggcggcccatagggactttccacatagggggcgttcaccatttcccagcataggggtggtgactcaatggcctttacccaagtacattgggtcaatgggaggtaagccaatgggtttttcccattactggcaagcacactgagtcaaatgggactttccactgggttttgcccaagtacattgggtcaatgggaggtgagccaatgggaaaaacccattgctgccaagtacactgactcaatagggactttccaatgggtttttccattgttggcaagcatataaggtcaatgtgggtgagtcaatagggactttccattgtattctgcccagtacataaggtcaatagggggtgaatcaacaggaaagtcccattggagccaagtacactgcgtcaatagggactttccattgggttttgcccagtacataaggtcaataggggatgagtcaatgggaaaaacccattggagccaagtacactgactcaatagggactttccattgggttttgcccagtacataaggtcaatagggggtgagtcaacaggaaagttccattggagccaagtacattgagtcaatagggactttccaatgggttttgcccagtacataaggtcaatgggaggtaagccaatgggtttttcccattactggcacgtatactgagtcattagggactttccaatgggttttgcccagtacataaggtcaataggggtgaatcaacaggaaagtcccattggagccaagtacactgagtcaatagggactttccattgggttttgcccagtacaaaaggtcaatagggggtgagtcaatgggtttttcccattattggcacgtacataaggtcaataggggtgagtcattgggtttttccagccaatttaattaaaacgccatgtactttcccaccattgacgtcaatgggctattgaaactaatgcaacgtgacctttaaacggtactttcccatagctgattaatgggaaagtaccgttctcgagccaatacacgtcaatgggaagtgaaagggcagccaaaacgtaacaccgccccggttttcccctggaaattccatattggcacgcattctattggctgagctgcgttctacgtgggtataagaggcgcgaccagcgtcggtaccgtcgcagtcttcggtctgaccaccgtagaacgcagagctcctcgctgcaggcggccgcatgggctccaaaccttctaccaggatcccagcacctctgatgctgatcacccggattatgctgatattgggctgtatccgtccgacaagctctcttgacggcaggcctcttgcagctgcaggaattgtagtaacaggagataaggcagtcaatgtatacacttcgtctcagacagggtcaatcatagtcaagttgctcccgaatatgcccagggataaggaggcgtgtgcaaaagccccattagaggcatataacagaacactgactactttgctcactcctcttggcgactccatccgcaagatccaagggtctgtgtccacatctggaggaggcaagcaaggccgcctgataggtgctgttattggcagtgtagctcttggggttgcaacagcggcacagataacagcagctgcggccctaatacaagccaaccagaatgccgccaacatcctccggcttaaggagagcattgctgcaaccaatgaagctgtgcatgaagtcaccgacggattatcacaactatcagtggcagttgggaagatgcagcagtttgtcaatgaccagtttaataatacggcgcgagaattggactgtataaaaatcacacaacaggttggtgtagaactcaacctatacctaactgaattgactacagtattcgggccacagatcacctcccctgcattaactcagctgaccatccaggcactttataatttagctggtggcaatatggattacttattaactaagttaggtatagggaacaatcaactcagctcgttaattggtagcggcctgatcactggttaccctatactgtatgactcacagactcaactcttgggcatacaagtgaatttaccctcagtcgggaacttaaataatatgcgtgccacctatttggagaccttatctgtaagtacaaccaaaggatatgcctcagcacttgtcccgaaagtagtgacacaagtcggttccgtgatagaagagcttgacacctcatactgtatagagtccgatctggatttatattgtactagaatagtgacattccccatgtccccaggtatttattcctgtttgagcggcaacacatcagcttgcatgtattcaaagactgaaggcgcactcactacgccgtatatggcccttaaaggctcagttattgccaattgtaaaataacaacatgtagatgtacagaccctcctggtatcatatcgcaaaattatggagaagctgtatccctgatagatagacattcgtgcaatgtcttatcattagacgggataactctaaggctcagtggggaatttgatgcaacttatcaaaagaacatctcaatactagattctcaagtcatcgtgacaggcaatcttgatatatcaactgaacttggaaacgtcaacaattcaatcagcaatgccttggataggttggcagaaagcaacagcaagctagaaaaagtcaatgtcagactaaccagcacatctgctctcattacctatattgttctaactgtcatttctctagttttcggtgcacttagtctggtgttagcgtgttacctgatgtacaaacagaaggcacaacaaaagaccttgctatggcttgggaataataccctcgatcagatgagagccactacaagagcatgagcggccgccccccccccccctaacgttactggccgaagccgcttggaataaggccggtgtgcgtttgtctatatgttattttccaccatattgccgtcttttggcaatgtgagggcccggaaacctggccctgtcttcttgacgagcattcctaggggtctttcccctctcgccaaaggaatgcaaggtctgttgaatgtcgtgaaggaagcagttcctctggaagcttcttgaagacaaacaacgtctgtagcgaccctttgcaggcagcggaaccccccacctggcgacaggtgcctctgcggccaaaagccacgtgtataagatacacctgcaaaggcggcacaaccccagtgccacgttgtgagttggatagttgtggaaagagtcaaatggctctcctcaagcgtattcaacaaggggctgaaggatgcccagaaggtaccccattgtatgggatctgatctggggcctcggtgcacatgctttacatgtgtttagtcgaggttaaaaaacgtctaggccccccgaaccacggggacgtggttttcctttgaaaaacacgatgataataccatgcaccgtcctcatctcagacggcactcgcgttactacgcgaaaggagaggtgcttaacaaacacatggattgcggtggaaaacggtgctgctcaggcgcagctgtattcactcttttctggacttgtgtcaggattatgcgggagcatatctgctttgtacgcaacgctatggaccgccatttatttttgaggaatgctttttggactatcgtactgctttcttccttcgctagccagagcaccgccgccgtcacgtacgactacattttaggccgtcgcgcgctcgacgcgctaaccataccggcggttggcccgtataacagatacctcactagggtatcaagaggctgcgacgttgtcgagctcaacccgatttctaacgtggacgacatgatatcggcggccaaagaaaaagagaaggggggccctttcgaggcctccgtcgtctggttctacgtgattaagggcgacgacggcgaggacaagtactgtccaatctatagaaaagagtacagggaatgtggcgacgtacaactgctatctgaatgcgccgttcaatctgcacagatgtgggcagtggactatgttcctagcacccttgtatcgcgaaatggcgcgggactgactatattctcccccactgctgcgctctctggccaatacttgctgaccctgaaaatcgggagatttgcgcaaacagctctcgtaactctagaagttaacgatcgctgtttaaagatcgggtcgcagcttaactttttaccgtcgaaatgctggacaacagaacagtatcagactggatttcaaggcgaacacctttatccgatcgcagacaccaatacacgacacgcggacgacgtatatcggggatacgaagatattctgcagcgctggaataatttgctgaggaaaaagaatcctagcgcgccagaccctcgtccagatagcgtcccgcaagaaattcccgctgtaaccaagaaagcggaagggcgcaccccggacgcagaaagcagcgaaaagaaggcccctccagaagactcggaggacgacatgcaggcagaggcttctggagaaaatcctgccgccctccccgaagacgacgaagtccccgaggacaccgagcacgatgatccaaactcggatcctgactattacaatgacatgcccgccgtgatcccggtggaggagactactaaaagttctaatgccgtctccatgcccatattcgcggcgttcgtagcctgcgcggtcgcgctcgtggggctactggtttggagcatcgtaaaatgcgcgcgtagctaagcggccgcggggatccagacatgataagatacattgatgagtttggacaaaccacaactagaatgcagtgaaaaaaatgctttatttgtgaaatttgtgatgctattgctttatttgtaaccattataagctgcaataaacaagttaacaacaacaattgcattcattttatgtttcaggttcagggggaggtgtgggaggtttttt

SEQ ID NO: 27 - DNA, 1857 bp, artificial sequence
  plasmid pHVTUS2SvgDwtsyn for vHVT406
  SV40 promoter (1)..(362)
  ILTV gD (379)..(1683)
  Syn Poly A (1695)..(1857)
gagctcggtacagcttggctgtggaatgtgtgtcagttagggtgtggaaagtccccaggctccccagcaggcagaagtatgcaaagcatgcatctcaattagtcagcaaccaggtgtggaaagtccccaggctccccagcaggcagaagtatgcaaagcatgcatctcaattagtcagcaaccatagtcccgcccctaactccgcccatcccgcccctaactccgcccagttccgcccattctccgccccatggctgactaattttttttatttatgcagaggccgaggccgcctcggcctctgagctattccagaagtagtgaggaggcttttttggaggcctaggcttttgcaaaaagctgcggccggccgccaccatgcaccgtcctcatctcagacggcactcgcgttactacgcgaaaggagaggtgcttaacaaacacatggattgcggtggaaaacggtgctgctcaggcgcagctgtattcactcttttctggacttgtgtcaggattatgcgggagcatatctgctttgtacgcaacgctatggaccgccatttatttttgaggaatgctttttggactatcgtactgctttcttccttcgctagccagagcaccgccgccgtcacgtacgactacattttaggccgtcgcgcgctcgacgcgctaaccataccggcggttggcccgtataacagatacctcactagggtatcaagaggctgcgacgttgtcgagctcaacccgatttctaacgtggacgacatgatatcggcggccaaagaaaaagagaaggggggccctttcgaggcctccgtcgtctggttctacgtgattaagggcgacgacggcgaggacaagtactgtccaatctatagaaaagagtacagggaatgtggcgacgtacaactgctatctgaatgcgccgttcaatctgcacagatgtgggcagtggactatgttcctagcacccttgtatcgcgaaatggcgcgggactgactatattctcccccactgctgcgctctctggccaatacttgctgaccctgaaaatcgggagatttgcgcaaacagctctcgtaactctagaagttaacgatcgctgtttaaagatcgggtcgcagcttaactttttaccgtcgaaatgctggacaacagaacagtatcagactggatttcaaggcgaacacctttatccgatcgcagacaccaatacacgacacgcggacgacgtatatcggggatacgaagatattctgcagcgctggaataatttgctgaggaaaaagaatcctagcgcgccagaccctcgtccagatagcgtcccgcaagaaattcccgctgtaaccaagaaagcggaagggcgcaccccggacgcagaaagcagcgaaaagaaggcccctccagaagactcggaggacgacatgcaggcagaggcttctggagaaaatcctgccgccctccccgaagacgacgaagtccccgaggacaccgagcacgatgatccaaactcggatcctgactattacaatgacatgcccgccgtgatcccggtggaggagactactaaaagttctaatgccgtctccatgcccatattcgcggcgttcgtagcctgcgcggtcgcgctcgtggggctactggtttggagcatcgtaaaatgcgcgcgtagctaatcgagcctagaggcaataaaatatctttattttcattacatctgtgtgttggttttttgtgtgaatcgatagtactaacatacgctctccatcaaaacaaaacgaaacaaaacaaactagcaaaataggctgtccccagtgcaagtgcaggtgccagaacatttctctctcgag